European Patent Application EP 4 613 763 A1, published September 10, 2025. Title: PROTEIN DERIVED FROM FIBRONECTIN TYPE III DOMAIN, AND USE THEREOF. Applicant: WOEI-JER CHUANG. Application EP. The sequence listing filed with the application follows.

SEQUENCE LISTING (28 sequences)

SEQ ID NO: 1 - protein, 94 aa, Homo sapiens
VSDVPRDLEVVAATPTSLLISWDAPAVTVRYYRITYGETGGNSPVQEFTVPGSKSTATISGLKPGVDYTITVYAVTGRGDSPASSKPISINYRT

SEQ ID NO: 2 - protein, 94 aa, synthetic construct
VSDVPRDLEVVAATPTSLLISWRHPHFPTRYYRITYGETGGNSPVQEFTVPLQPPTATISGLKPGVDYTITVYAVTDGRNGRLLSIPISINYRT

SEQ ID NO: 3 - protein, 101 aa, synthetic construct
MVSDVPRDLEVVEASPTSIQISWRHPHFPTRYYRITYGETGGNSPVQEFTVPLQPPTATISGLKPGVDYTITVYAVTDGRNGRLLSIPISINYRTHHHHHH

SEQ ID NO: 4 - protein, 94 aa, synthetic construct
VSDVPRDCEVVAATPTSLLISCRHPHFPTRYYRITYGETGGNSPVQEFTVPLQPPTATISGLKPGVDYTITVYAVTDGRNGRLLSIPISINYRT

SEQ ID NO: 5 - protein, 94 aa, synthetic construct
VSDVPRDLEVVAATPTCLLISWRHPHFPTRYYRITYGETGGNSPVQEFTVPLQPPTATICGLKPGVDYTITVYAVTDGRNGRLLSIPISINYRT

SEQ ID NO: 6 - protein, 94 aa, synthetic construct
VSDVPRDLEVVAATPTSLLISWRHPHFPTRYYRITYGECGGNSPVQEFTVPLQPPTATISGLKPGVCYTITVYAVTDGRNGRLLSIPISINYRT

SEQ ID NO: 7 - protein, 94 aa, synthetic construct
VSDVPRDLEVVAATPTSLLISWRHPHFPTRYYRITYGETGGNSPVQEFTVPLQPPTATISGLCPGCDYTITVYAVTDGRNGRLLSIPISINYRT

SEQ ID NO: 8 - protein, 94 aa, synthetic construct
VSDVPRDLEVVAATPTSLCISWRHPHFPTRYYRITYGETGGNSPVQEFTVPLQPPTACISGLKPGVDYTITVYAVTDGRNGRLLSIPISINYRT

SEQ ID NO: 9 - protein, 94 aa, synthetic construct
VSDVPRDLEVVAATPTSLLISWRHPHFPTRYYRCTYGETGGNSPVQECTVPLQPPTATISGLKPGVDYTITVYAVTDGRNGRLLSIPISINYRT

SEQ ID NO: 10 - protein, 94 aa, synthetic construct
VSDVPRDLEVVAATPTSLLISWRHPHFPTRYYRITCGETGGNSPVQEFTVPLQPPTATISGLKPGVDYTCTVYAVTDGRNGRLLSIPISINYRT

SEQ ID NO: 11 - protein, 94 aa, synthetic construct
VSDVPRDCEVVAATPTSLLISWRHPHFPTRYYRITYGETGGNSPVQEFTVPLQPPTATISGLKPGVDYTITVYAVTDGRNGRLLSIPICINYRT

SEQ ID NO: 12 - protein, 94 aa, synthetic construct
VSDVPRDLEVVAATPTSLLISWRHPHFPTRYYRICYGETGGNSPCQEFTVPLQPPTATISGLKPGVDYTITVYAVTDGRNGRLLSIPISINYRT

SEQ ID NO: 13 - protein, 94 aa, synthetic construct
VSDVPRDLEVVAATPTSLLISWRHPHFPTRYYRITYCETGGNSPCQEFTVPLQPPTATISGLKPGVDYTITVYAVTDGRNGRLLSIPISINYRT

SEQ ID NO: 14 - protein, 94 aa, synthetic construct
VSDVPRDLEVVAATPTSLLISWRHPHFPTRYYRITYGETGGNSPVQEFTVPLQPPTATISGLKPGVCYTITVYAVTDGRNGRLLSIPISICYRT

SEQ ID NO: 15 - protein, 94 aa, synthetic construct
VSDVPRDCEVVAATPTCLLISWRHPHFPTRYYRITYGETGGNSPVQEFTVPLQPPTATICGLKPGVDYTITVYAVTDGRNGRLLSIPICINYRT

SEQ ID NO: 16 - protein, 94 aa, synthetic construct
VSDVPRDCEVVAATPTSLLISWRHPHFPTRYYRITYGECGGNSPVQEFTVPLQPPTATISGLKPGVCYTITVYAVTDGRNGRLLSIPICINYRT

SEQ ID NO: 17 - protein, 94 aa, synthetic construct
VSDVPRDCEVVEASPTSIQISCRHPHFPTRYYRITYGETGGNSPVQEFTVPLQPPTATISGLKPGVDYTITVYAVTDGRNGRLLSIPISINYRT

SEQ ID NO: 18 - protein, 94 aa, synthetic construct
VSDVPRDLEVVEASPTCIQISWRHPHFPTRYYRITYGETGGNSPVQEFTVPLQPPTATICGLKPGVDYTITVYAVTDGRNGRLLSIPISINYRT

SEQ ID NO: 19 - protein, 94 aa, synthetic construct
VSDVPRDLEVVEASPTSIQISWRHPHFPTRYYRITYGECGGNSPVQEFTVPLQPPTATISGLKPGVCYTITVYAVTDGRNGRLLSIPISINYRT

SEQ ID NO: 20 - protein, 94 aa, synthetic construct
VSDVPRDLEVVEASPTSIQISWRHPHFPTRYYRITYGETGGNSPVQEFTVPLQPPTATISGLCPGCDYTITVYAVTDGRNGRLLSIPISINYRT

SEQ ID NO: 21 - protein, 94 aa, synthetic construct
VSDVPRDLEVVEASPTSIQISWRHPHFPTRYYRCTYGETGGNSPVQECTVPLQPPTATISGLKPGVDYTITVYAVTDGRNGRLLSIPISINYRT

SEQ ID NO: 22 - protein, 94 aa, synthetic construct
VSDVPRDLEVVEASPTSIQISWRHPHFPTRYYRITCGETGGNSPVQEFTVPLQPPTATISGLKPGVDYTCTVYAVTDGRNGRLLSIPISINYRT

SEQ ID NO: 23 - protein, 94 aa, synthetic construct
VSDVPRDCEVVEASPTSIQISWRHPHFPTRYYRITYGETGGNSPVQEFTVPLQPPTATISGLKPGVDYTITVYAVTDGRNGRLLSIPICINYRT

SEQ ID NO: 24 - protein, 94 aa, unidentified
VSDVPRDLEVVEASPTSIQISWRHPHFPTRYYRICYGETGGNSPCQEFTVPLQPPTATISGLKPGVDYTITVYAVTDGRNGRLLSIPISINYRT

SEQ ID NO: 25 - protein, 94 aa, synthetic construct
VSDVPRDLEVVEASPTSIQISWRHPHFPTRYYRITYCETGGNSPCQEFTVPLQPPTATISGLKPGVDYTITVYAVTDGRNGRLLSIPISINYRT

SEQ ID NO: 26 - protein, 94 aa, synthetic construct
VSDVPRDLEVVEASPTSIQISWRHPHFPTRYYRITYGETGGNSPVQEFTVPLQPPTATISGLKPGVCYTITVYAVTDGRNGRLLSIPISICYRT

SEQ ID NO: 27 - protein, 94 aa, synthetic construct
VSDVPRDCEVVEASPTCIQISWRHPHFPTRYYRITYGETGGNSPVQEFTVPLQPPTATICGLKPGVDYTITVYAVTDGRNGRLLSIPICINYRT

SEQ ID NO: 28 - protein, 94 aa, synthetic construct
VSDVPRDCEVVEASPTSIQISWRHPHFPTRYYRITYGECGGNSPVQEFTVPLQPPTATISGLKPGVCYTITVYAVTDGRNGRLLSIPICINYRT